European Patent Application EP 4 653 869 A1, published November 26, 2025. Title: MOLECULES MIMICKING INTERLEUKIN 34 BONE REGULATION ACTIVITY BASED ON THE BINDING OF IL-34 TO BONE MORPHOGENETIC PROTEINS, METHOD OF SCREENING AND PHARMACEUTICAL COMPOSITION. Applicant: Nantes Universite. The sequence listing filed with the application follows.

SEQUENCE LISTING (2 sequences)

SEQ ID NO: 1 - protein, 10 aa, Homo sp.
KLQYRSRQYM

SEQ ID NO: 2 - protein, 17 aa, Homo sp.
EGHPSWKYLQEVETLLL